European Patent Specification EP 3 943 093 B1, published May 7, 2025. Title: USE OF PASTEURIZED AKKERMANSIA FOR TREATING METABOLIC DISORDERS. Applicant: Université catholique de Louvain Wageningen Universiteit. The sequence listing filed with the application follows.

SEQUENCE LISTING (8 sequences)

SEQ ID NO: 1 - DNA, 23 bp, Artificial Sequence
  Primer RPL-19 Forward
gaaggtcaaagggaatgtgttca

SEQ ID NO: 2 - DNA, 21 bp, Artificial Sequence
  Primer RPL-19 Reverse
ccttgtctgccttcagcttgt

SEQ ID NO: 3 - DNA, 19 bp, Artificial Sequence
  Primer Ocln Forward
atgtccggccgatgctctc

SEQ ID NO: 4 - DNA, 23 bp, Artificial Sequence
  Primer Ocln Reverse
tttggctgctcttgggtctgtat

SEQ ID NO: 5 - DNA, 22 bp, Artificial Sequence
  Primer Cldn3 Forward
tcatcggcagcagcatcatcac

SEQ ID NO: 6 - DNA, 22 bp, Artificial Sequence
  Primer Cldn3 Reverse
acgatggtgatcttggccttgg

SEQ ID NO: 7 - DNA, 27 bp, Artificial Sequence
  Primer Lyz1 Forward
gccaaggtctacaatcgttgtgagttg

SEQ ID NO: 8 - DNA, 23 bp, Artificial Sequence
  Primer Lyz1 Reverse
cagtcagccagcttgacaccacg